European Patent Specification EP 3 854 875 B1, published January 14, 2026. Title: Human monoclonal antibody specifically binding to human HMGB1, and pharmaceutical composition for treating or preventing Alzheimer's disease comprising the same. Applicant: NATIONAL UNIVERSITY CORPORATION TOKYO MEDICAL AND DENTAL UNIVERSITY. The sequence listing filed with the application follows.

SEQUENCE LISTING (42 sequences)

SEQ ID NO: 1 - protein, 457 aa, Artificial
  #127 heavy chain (variable region and constant region)
  MISC_FEATURE: Inventor:OKAZAWA, Hitoshi
EVQLLESGGGLVQPGGSLRLSCAASGFTFSSYAMSWVRQAPGKGLEWVSAISGSGGSTYYADSVKGRFTISRDNSKNTLYLQMNSLRAEDTAVYYCTKDGYSSSWDYYYYYYGMDVWGQGTTVTVSSASTKGPSVFPLAPSSKSTSGGTAALGCLVKDYFPEPVTVSWNSGALTSGVHTFPAVLQSSGLYSLSSVVTVPSSSLGTQTYICNVNHKPSNTKVDKKVEPKSCDKTHTCPPCPAPELLGGPSVFLFPPKPKDTLMISRTPEVTCVVVDVSHEDPEVKFNWYVDGVEVHNAKTKPREEQYNSTYRVVSVLTVLHQDWLNGKEYKCKVSNKALPAPIEKTISKAKGQPREPQVYTLPPSREEMTKNQVSLTCLVKGFYPSDIAVEWESNGQPENNYKTTPPVLDSDGSFFLYSKLTVDKSRWQQGNVFSCSVMHEALHNHYTQKSLSLSPGK

SEQ ID NO: 2 - protein, 127 aa, Artificial
  #127 heavy chain variable region
EVQLLESGGGLVQPGGSLRLSCAASGFTFSSYAMSWVRQAPGKGLEWVSAISGSGGSTYYADSVKGRFTISRDNSKNTLYLQMNSLRAEDTAVYYCTKDGYSSSWDYYYYYYGMDVWGQGTTVTVSS

SEQ ID NO: 3 - protein, 5 aa, Artificial
  #127 heavy chain CDR1
SYAMS

SEQ ID NO: 4 - protein, 17 aa, Artificial
  #127 heavy chain CDR2
AISGSGGSTYYADSVKG

SEQ ID NO: 5 - protein, 18 aa, Artificial
  #127 heavy chain CDR3
DGYSSSWDYYYYYYGMDV

SEQ ID NO: 6 - protein, 213 aa, Artificial
  #127 light chain (variable region and constant region)
DIQMTQSPSSLSASVGDRVTITCRASQSVSSYLAWYQQKPGKAPKLLIYEASNLQAGVPSRFSGSGSGTDFTLTINSLQPEDFATYYCLQHNSNPLTFGQGTKLEIKTVAAPSVFIFPPSDEQLKSGTASVVCLLNNFYPREAKVQWKVDNALQSGNSQESVTEQDSKDSTYSLSSTLTLSKADYEKHKVYACEVTHQGLSSPVTKSFNRGEC

SEQ ID NO: 7 - protein, 107 aa, Artificial
  #127 light chain variable region
DIQMTQSPSSLSASVGDRVTITCRASQSVSSYLAWYQQKPGKAPKLLIYEASNLQAGVPSRFSGSGSGTDFTLTINSLQPEDFATYYCLQHNSNPLTFGQGTKLEIK

SEQ ID NO: 8 - protein, 11 aa, Artificial
  #127 light chain CDR1
RASQSVSSYLA

SEQ ID NO: 9 - protein, 7 aa, Artificial
  #127 light chain CDR2
EASNLQA

SEQ ID NO: 10 - protein, 9 aa, Artificial
  #127 light chain CDR3
LQHNSNPLT

SEQ ID NO: 11 - protein, 445 aa, Artificial
  #129 heavy chain (variable region and constant region)
EVQLLESGGGLVQPGGSLRLSCAASGFTFSSYAMSWVRQAPGKGLEWVSDISGSGGSTYYADSVKGRFTISRDNSKNTLYLQMNSLRAEDTAVYYCARGYGMDVWGQGTMVTVSSASTKGPSVFPLAPSSKSTSGGTAALGCLVKDYFPEPVTVSWNSGALTSGVHTFPAVLQSSGLYSLSSVVTVPSSSLGTQTYICNVNHKPSNTKVDKKVEPKSCDKTHTCPPCPAPELLGGPSVFLFPPKPKDTLMISRTPEVTCVVVDVSHEDPEVKFNWYVDGVEVHNAKTKPREEQYNSTYRVVSVLTVLHQDWLNGKEYKCKVSNKALPAPIEKTISKAKGQPREPQVYTLPPSREEMTKNQVSLTCLVKGFYPSDIAVEWESNGQPENNYKTTPPVLDSDGSFFLYSKLTVDKSRWQQGNVFSCSVMHEALHNHYTQKSLSLSPGK

SEQ ID NO: 12 - protein, 115 aa, Artificial
  #129 heavy chain variable region
EVQLLESGGGLVQPGGSLRLSCAASGFTFSSYAMSWVRQAPGKGLEWVSDISGSGGSTYYADSVKGRFTISRDNSKNTLYLQMNSLRAEDTAVYYCARGYGMDVWGQGTMVTVSS

SEQ ID NO: 13 - protein, 5 aa, Artificial
  #129 heavy chain CDR1
SYAMS

SEQ ID NO: 14 - protein, 17 aa, Artificial
  #129 heavy chain CDR2
DISGSGGSTYYADSVKG

SEQ ID NO: 15 - protein, 6 aa, Artificial
  #129 heavy chain CDR3
GYGMDV

SEQ ID NO: 16 - protein, 213 aa, Artificial
  #129 light chain (variable region and constant region)
DIQMTQSPSSLSASVGDRVTITCRASQSVTNYLAWYQQKPGKAPKLLIYGASILETGVPSRFSGSGSGTDFTLTINSLQPEDFATYYCLQHNSTPLTFGQGTKLEIKTVAAPSVFIFPPSDEQLKSGTASVVCLLNNFYPREAKVQWKVDNALQSGNSQESVTEQDSKDSTYSLSSTLTLSKADYEKHKVYACEVTHQGLSSPVTKSFNRGEC

SEQ ID NO: 17 - protein, 107 aa, Artificial
  #129 light chain variable region
DIQMTQSPSSLSASVGDRVTITCRASQSVTNYLAWYQQKPGKAPKLLIYGASILETGVPSRFSGSGSGTDFTLTINSLQPEDFATYYCLQHNSTPLTFGQGTKLEIK

SEQ ID NO: 18 - protein, 11 aa, Artificial
  #129 light chain CDR1
RASQSVTNYLA

SEQ ID NO: 19 - protein, 7 aa, Artificial
  #129 light chain CDR2
GASILET

SEQ ID NO: 20 - protein, 9 aa, Artificial
  #129 light chain CDR3
LQHNSTPLT

SEQ ID NO: 21 - protein, 444 aa, Artificial
  #213-001 heavy chain (variable region and constant region)
EVQLVQSGAEVKKPGSSVKVSCKASGGTFSSYAISWVRQAPGQGLEWMGGIIPIFGRANYAQKFQGRVTITADESTSTAYMELSSLRSEDTAVYYCASLVTDYWGQGTLVTVSSASTKGPSVFPLAPSSKSTSGGTAALGCLVKDYFPEPVTVSWNSGALTSGVHTFPAVLQSSGLYSLSSVVTVPSSSLGTQTYICNVNHKPSNTKVDKKVEPKSCDKTHTCPPCPAPELLGGPSVFLFPPKPKDTLMISRTPEVTCVVVDVSHEDPEVKFNWYVDGVEVHNAKTKPREEQYNSTYRVVSVLTVLHQDWLNGKEYKCKVSNKALPAPIEKTISKAKGQPREPQVYTLPPSREEMTKNQVSLTCLVKGFYPSDIAVEWESNGQPENNYKTTPPVLDSDGSFFLYSKLTVDKSRWQQGNVFSCSVMHEALHNHYTQKSLSLSPGK

SEQ ID NO: 22 - protein, 114 aa, Artificial
  #213-001 heavy chain variable region
EVQLVQSGAEVKKPGSSVKVSCKASGGTFSSYAISWVRQAPGQGLEWMGGIIPIFGRANYAQKFQGRVTITADESTSTAYMELSSLRSEDTAVYYCASLVTDYWGQGTLVTVSS

SEQ ID NO: 23 - protein, 5 aa, Artificial
  #213-001 heavy chain CDR1
SYAIS

SEQ ID NO: 24 - protein, 17 aa, Artificial
  #213-001 heavy chain CDR2
GIIPIFGRANYAQKFQG

SEQ ID NO: 25 - protein, 5 aa, Artificial
  #213-001 heavy chain CDR3
LVTDY

SEQ ID NO: 26 - protein, 213 aa, Artificial
  #213-001 light chain (variable region and constant region)
DIQMTQSPSSLSASTGDRVTITCRASQGISSYLAWYQQKPGKAPKLLIYAASTLQSGVPSRFSGSGSGTDFTLTISSLQPEDFATYYCQQANSFPITFGQGTRLEIKTVAAPSVFIFPPSDEQLKSGTASVVCLLNNFYPREAKVQWKVDNALQSGNSQESVTEQDSKDSTYSLSSTLTLSKADYEKHKVYACEVTHQGLSSPVTKSFNRGEC

SEQ ID NO: 27 - protein, 107 aa, Artificial
  #213-001 light chain variable region
DIQMTQSPSSLSASTGDRVTITCRASQGISSYLAWYQQKPGKAPKLLIYAASTLQSGVPSRFSGSGSGTDFTLTISSLQPEDFATYYCQQANSFPITFGQGTRLEIK

SEQ ID NO: 28 - protein, 11 aa, Artificial
  #213-001 light chain CDR1
RASQGISSYLA

SEQ ID NO: 29 - protein, 7 aa, Artificial
  #213-001 light chain CDR2
AASTLQS

SEQ ID NO: 30 - protein, 9 aa, Artificial
  #213-001 light chain CDR3
QQANSFPIT

SEQ ID NO: 31 - protein, 444 aa, Artificial
  #213-012 heavy chain (variable region and constant region)
EVQLVQSGAEVKKPGSSVKVSCKASGGTFSSYAISWVRQAPGQGLEWMGGIIPIFGTANYAQKFQGRVTITADESTSTAYMELSSLRSEDTAVYYCASLVTDYWGQGTLVTVSSASTKGPSVFPLAPSSKSTSGGTAALGCLVKDYFPEPVTVSWNSGALTSGVHTFPAVLQSSGLYSLSSVVTVPSSSLGTQTYICNVNHKPSNTKVDKKVEPKSCDKTHTCPPCPAPELLGGPSVFLFPPKPKDTLMISRTPEVTCVVVDVSHEDPEVKFNWYVDGVEVHNAKTKPREEQYNSTYRVVSVLTVLHQDWLNGKEYKCKVSNKALPAPIEKTISKAKGQPREPQVYTLPPSREEMTKNQVSLTCLVKGFYPSDIAVEWESNGQPENNYKTTPPVLDSDGSFFLYSKLTVDKSRWQQGNVFSCSVMHEALHNHYTQKSLSLSPGK

SEQ ID NO: 32 - protein, 114 aa, Artificial
  #213-012 heavy chain variable region
EVQLVQSGAEVKKPGSSVKVSCKASGGTFSSYAISWVRQAPGQGLEWMGGIIPIFGTANYAQKFQGRVTITADESTSTAYMELSSLRSEDTAVYYCASLVTDYWGQGTLVTVSS

SEQ ID NO: 33 - protein, 5 aa, Artificial
  #213-012 heavy chain CDR1
SYAIS

SEQ ID NO: 34 - protein, 17 aa, Artificial
  #213-012 heavy chain CDR2
GIIPIFGTANYAQKFQG

SEQ ID NO: 35 - protein, 5 aa, Artificial
  #213-012 heavy chain CDR3
LVTDY

SEQ ID NO: 36 - protein, 213 aa, Artificial; identical to SEQ ID NO: 26
  #213-012 light chain (variable region and constant region)

SEQ ID NO: 37 - protein, 107 aa, Artificial; identical to SEQ ID NO: 27
  #213-012 light chain variable region

SEQ ID NO: 38 - protein, 11 aa, Artificial
  #213-012 light chain CDR1
RASQGISSYLA

SEQ ID NO: 39 - protein, 7 aa, Artificial
  #213-012 light chain CDR2
AASTLQS

SEQ ID NO: 40 - protein, 9 aa, Artificial
  #213-012 light chain CDR3
QQANSFPIT

SEQ ID NO: 41 - protein, 330 aa, Artificial
  the present invention antibody heavy chain constant region
ASTKGPSVFPLAPSSKSTSGGTAALGCLVKDYFPEPVTVSWNSGALTSGVHTFPAVLQSSGLYSLSSVVTVPSSSLGTQTYICNVNHKPSNTKVDKKVEPKSCDKTHTCPPCPAPELLGGPSVFLFPPKPKDTLMISRTPEVTCVVVDVSHEDPEVKFNWYVDGVEVHNAKTKPREEQYNSTYRVVSVLTVLHQDWLNGKEYKCKVSNKALPAPIEKTISKAKGQPREPQVYTLPPSREEMTKNQVSLTCLVKGFYPSDIAVEWESNGQPENNYKTTPPVLDSDGSFFLYSKLTVDKSRWQQGNVFSCSVMHEALHNHYTQKSLSLSPGK

SEQ ID NO: 42 - protein, 106 aa, Artificial
  the present invention antibody light chain constant region (kappa chain)
TVAAPSVFIFPPSDEQLKSGTASVVCLLNNFYPREAKVQWKVDNALQSGNSQESVTEQDSKDSTYSLSSTLTLSKADYEKHKVYACEVTHQGLSSPVTKSFNRGEC